European Patent Specification EP 3 828 285 B1, published December 13, 2023. Title: TRANSPOSITION INTO NATIVE CHROMATIN FOR PERSONAL EPIGENOMICS. Applicant: THE BOARD OF TRUSTEES OF THE LELAND STANFORD JUNIOR UNIVERSITY. The sequence listing filed with the application follows.

SEQUENCE LISTING (25 sequences)

SEQ ID NO: 1 - DNA, 50 bp, Artificial Sequence
  synthetic polynucleotide
aatgatacggcgaccaccgagatctacactcgtcggcagcgtcagatgtg

SEQ ID NO: 2 - DNA, 53 bp, Artificial sequence
  synthetic polynucleotide
caagcagaagacggcatacgagattcgccttagtctcgtgggctcggagatgt

SEQ ID NO: 3 - DNA, 53 bp, Artificial sequence
  synthetic polynucleotide
caagcagaagacggcatacgagatctagtacggtctcgtgggctcggagatgt

SEQ ID NO: 4 - DNA, 53 bp, Artificial sequence
  synthetic polynucleotide
caagcagaagacggcatacgagatttctgcctgtctcgtgggctcggagatgt

SEQ ID NO: 5 - DNA, 53 bp, Artificial sequence
  synthetic polynucleotide
caagcagaagacggcatacgagatgctcaggagtctcgtgggctcggagatgt

SEQ ID NO: 6 - DNA, 53 bp, Artificial sequence
  synthetic polynucleotide
caagcagaagacggcatacgagataggagtccgtctcgtgggctcggagatgt

SEQ ID NO: 7 - DNA, 53 bp, Artificial sequence
  synthetic polynucleotide
caagcagaagacggcatacgagatcatgcctagtctcgtgggctcggagatgt

SEQ ID NO: 8 - DNA, 53 bp, Artificial sequence
  synthetic polynucleotide
caagcagaagacggcatacgagatgtagagaggtctcgtgggctcggagatgt

SEQ ID NO: 9 - DNA, 53 bp, Artificial sequence
  synthetic polynucleotide
caagcagaagacggcatacgagatcctctctggtctcgtgggctcggagatgt

SEQ ID NO: 10 - DNA, 53 bp, Artificial sequence
  synthetic polynucleotide
caagcagaagacggcatacgagatagcgtagcgtctcgtgggctcggagatgt

SEQ ID NO: 11 - DNA, 53 bp, Artificial sequence
  synthetic polynucleotide
caagcagaagacggcatacgagatcagcctcggtctcgtgggctcggagatgt

SEQ ID NO: 12 - DNA, 53 bp, Artificial sequence
  synthetic polynucleotide
caagcagaagacggcatacgagattgcctcttgtctcgtgggctcggagatgt

SEQ ID NO: 13 - DNA, 53 bp, Artificial sequence
  synthetic polynucleotide
caagcagaagacggcatacgagattcctctacgtctcgtgggctcggagatgt

SEQ ID NO: 14 - DNA, 53 bp, Artificial sequence
  synthetic polynucleotide
caagcagaagacggcatacgagatatcacgacgtctcgtgggctcggagatgt

SEQ ID NO: 15 - DNA, 53 bp, Artificial sequence
  synthetic polynucleotide
caagcagaagacggcatacgagatacagtggtgtctcgtgggctcggagatgt

SEQ ID NO: 16 - DNA, 53 bp, Artificial sequence
  synthetic polynucleotide
caagcagaagacggcatacgagatcagatccagtctcgtgggctcggagatgt

SEQ ID NO: 17 - DNA, 53 bp, Artificial sequence
  synthetic polynucleotide
caagcagaagacggcatacgagatacaaacgggtctcgtgggctcggagatgt

SEQ ID NO: 18 - DNA, 53 bp, Artificial sequence
  synthetic polynucleotide
caagcagaagacggcatacgagatacccagcagtctcgtgggctcggagatgt

SEQ ID NO: 19 - DNA, 53 bp, Artificial sequence
  synthetic polynucleotide
caagcagaagacggcatacgagataacccctcgtctcgtgggctcggagatgt

SEQ ID NO: 20 - DNA, 53 bp, Artificial sequence
  synthetic polynucleotide
caagcagaagacggcatacgagatcccaacctgtctcgtgggctcggagatgt

SEQ ID NO: 21 - DNA, 53 bp, Artificial sequence
  synthetic polynucleotide
caagcagaagacggcatacgagatcaccacacgtctcgtgggctcggagatgt

SEQ ID NO: 22 - DNA, 53 bp, Artificial sequence
  synthetic polynucleotide
caagcagaagacggcatacgagatgaaacccagtctcgtgggctcggagatgt

SEQ ID NO: 23 - DNA, 53 bp, Artificial sequence
  synthetic polynucleotide
caagcagaagacggcatacgagattgtgaccagtctcgtgggctcggagatgt

SEQ ID NO: 24 - DNA, 53 bp, Artificial sequence
  synthetic polynucleotide
caagcagaagacggcatacgagatagggtcaagtctcgtgggctcggagatgt

SEQ ID NO: 25 - DNA, 53 bp, Artificial sequence
  synthetic polynucleotide
caagcagaagacggcatacgagataggagtgggtctcgtgggctcggagatgt